European Patent Application EP 4 299 760 A2, published January 3, 2024. Title: PROBES FOR IMPROVED MELT DISCRIMINATION AND MULTIPLEXING IN NUCLEIC ACID ASSAYS. Applicant: Luminex Corporation. The sequence listing filed with the application follows.

SEQUENCE LISTING (31 sequences)

SEQ ID NO: 1 - DNA, 29 bp, synthetic construct
  source 1..29: mol_type = other DNA
atatcagtcattgcccaaaccgcaatgac

SEQ ID NO: 2 - DNA, 34 bp, synthetic construct
  source 1..34: mol_type = other DNA
atatcagtcattgcccaaaaaaaaccgcaatgac

SEQ ID NO: 3 - DNA, 27 bp, synthetic construct
  source 1..27: mol_type = other DNA
atatcagtcttgcccaaaccgcaagac

SEQ ID NO: 4 - DNA, 32 bp, synthetic construct
  source 1..32: mol_type = other DNA
atatcagtcttgcccaaaaaaaaccgcaagac

SEQ ID NO: 5 - DNA, 31 bp, synthetic construct
  source 1..31: mol_type = other DNA
atatcagtcaattgcccaaaccgcaattgac

SEQ ID NO: 6 - DNA, 36 bp, synthetic construct
  source 1..36: mol_type = other DNA
atatcagtcaattgcccaaaaaaaaccgcaattgac

SEQ ID NO: 7 - DNA, 29 bp, synthetic construct
  source 1..29: mol_type = other DNA
atatcagtcaagtgccaaacccacttgac

SEQ ID NO: 8 - DNA, 34 bp, synthetic construct
  source 1..34: mol_type = other DNA
atatcagtcaagtgccaaaaaaaacccacttgac

SEQ ID NO: 9 - DNA, 25 bp, synthetic construct
  source 1..25: mol_type = other DNA
atatcaggtcagccaaaccctgacc

SEQ ID NO: 10 - DNA, 25 bp, synthetic construct
  source 1..25: mol_type = other DNA
atatcagtctgcccaaaccgcagac

SEQ ID NO: 11 - DNA, 25 bp, synthetic construct
  source 1..25: mol_type = other DNA
atatcagtctgcccaaaccgcagac

SEQ ID NO: 12 - DNA, 66 bp, synthetic construct
  misc_feature 1..41: note = DNA
  misc_feature 42: note = RNA
  misc_feature 43..66: note = DNA
  source 1..66: mol_type = other DNA
atatcagtcattgcccaaaaaaaaaaaaaaaaccgcaatgaccatgagacagtatagtagcgctga

SEQ ID NO: 13 - DNA, 58 bp, synthetic construct
  misc_feature 1..34: note = DNA
  misc_feature 35: note = RNA
  misc_feature 36..58: note = DNA
  source 1..58: mol_type = other DNA
atatcagtcattgcccaaaaaaaaccgcaatgaccatgagacagtatagtagcgctga

SEQ ID NO: 14 - DNA, 60 bp, synthetic construct
  misc_feature 1..36: note = DNA
  misc_feature 37: note = RNA
  misc_feature 38..60: note = DNA
  source 1..60: mol_type = other DNA
atatcagtcatgtgcccaaaaaaaaccgcacatgaccatgagacagtatagtagcgctga

SEQ ID NO: 15 - DNA, 60 bp, synthetic construct
  misc_feature 1..36: note = DNA
  misc_feature 37: note = RNA
  misc_feature 38..60: note = DNA
  source 1..60: mol_type = other DNA
atatcagtcatttgcccaaaaaaaaccgcaaatgaccatgagacagtatagtagcgctga

SEQ ID NO: 16 - DNA, 60 bp, synthetic construct
  misc_feature 1..36: note = DNA
  misc_feature 37: note = RNA
  misc_feature 38..60: note = DNA
  source 1..60: mol_type = other DNA
atatcagtcaattgcccaaaaaaaaccgcaattgaccatgagacagtatagtagcgctga

SEQ ID NO: 17 - DNA, 58 bp, synthetic construct
  misc_feature 1..34: note = DNA
  misc_feature 35: note = RNA
  misc_feature 36..58: note = DNA
  source 1..58: mol_type = other DNA
atatcagtcattgaccaaaaaaaacctcaatgaccatgagacagtatagtagcgctga

SEQ ID NO: 18 - DNA, 58 bp, synthetic construct
  misc_feature 1..34: note = DNA
  misc_feature 35: note = RNA
  misc_feature 36..58: note = DNA
  source 1..58: mol_type = other DNA
atatcagtcattacccaaaaaaaaccgtaatgaccatgagacagtatagtagcgctga

SEQ ID NO: 19 - DNA, 60 bp, synthetic construct
  misc_feature 1..36: note = DNA
  misc_feature 37: note = RNA
  misc_feature 38..60: note = DNA
  source 1..60: mol_type = other DNA
atatcagtcatgtacccaaaaaaaaccgtacatgaccatgagacagtatagtagcgctga

SEQ ID NO: 20 - DNA, 62 bp, synthetic construct
  misc_feature 1..38: note = DNA
  misc_feature 39: note = RNA
  misc_feature 40..62: note = DNA
  source 1..62: mol_type = other DNA
atatcagtcattgtacccaaaaaaaaccgtacaatgaccatgagacagtatagtagcgctga

SEQ ID NO: 21 - DNA, 70 bp, synthetic construct
  misc_feature 1..46: note = DNA
  misc_feature 47: note = RNA
  misc_feature 48..70: note = DNA
  source 1..70: mol_type = other DNA
atatcagtcaatgtgcccaaaaaaaaaaaaaaaaccgcacattgaccatgagacagtatagtagcgctga

SEQ ID NO: 22 - DNA, 23 bp, synthetic construct
  source 1..23: mol_type = other DNA
gaagcatttgaaatagcagaagg

SEQ ID NO: 23 - DNA, 23 bp, synthetic construct
  source 1..23: mol_type = other DNA
cacagagcgttcctagttttact

SEQ ID NO: 24 - DNA, 21 bp, synthetic construct
  source 1..21: mol_type = other DNA
atatcagtcatttgcccaaaa

SEQ ID NO: 25 - DNA, 38 bp, synthetic construct
  misc_feature 1..14: note = DNA
  misc_feature 15: note = RNA
  misc_feature 16..38: note = DNA
  source 1..38: mol_type = other DNA
aaaccgcaaatgaccatgagacagtatagtagcgctga

SEQ ID NO: 26 - DNA, 24 bp, synthetic construct
  source 1..24: mol_type = other DNA
caaaaaaaagtcatgttaccaaaa

SEQ ID NO: 27 - DNA, 34 bp, synthetic construct
  misc_feature 1..14: note = DNA
  misc_feature 15: note = RNA
  misc_feature 16..34: note = DNA
  source 1..34: mol_type = other DNA
aaacctaacatgaccatgagacagtatagtagcg

SEQ ID NO: 28 - DNA, 32 bp, synthetic construct
  source 1..32: mol_type = other DNA
catatcatcatcatctcattttaggcccaaaa

SEQ ID NO: 29 - DNA, 33 bp, synthetic construct
  misc_feature 1..14: note = DNA
  misc_feature 15: note = RNA
  misc_feature 16..33: note = DNA
  source 1..33: mol_type = other DNA
aaaccgcctaaaatccccttagtcagaggtgac

SEQ ID NO: 30 - DNA, 36 bp, synthetic construct
  source 1..36: mol_type = other DNA
ctccatcctcctcctcctctctcttcgagaccaaaa

SEQ ID NO: 31 - DNA, 26 bp, synthetic construct
  misc_feature 1..13: note = DNA
  misc_feature 14: note = RNA
  misc_feature 15..26: note = DNA
  source 1..26: mol_type = other DNA
aaacctctcgaagcgtcctgtccggc